European Patent Application EP 4 725 507 A1, published April 15, 2026. Title: 多肽偶联物、包含所述多肽偶联物的药物组合物及其用途. Applicant: 南京安吉生物科技有限公司. Application CN. The sequence listing filed with the application follows.

SEQUENCE LISTING (1 sequence)

SEQ ID NO: 1 - protein, 7 aa, synthetic construct
RSPYANS